European Patent Application EP 4 471 052 A1, published December 4, 2024. Title: 一种融合表达Tau-4R蛋白的大肠杆菌工程菌株. Applicant: 元本(珠海横琴)生物科技有限公司. The sequence listing filed with the application follows.

SEQUENCE LISTING (4 sequences)

SEQ ID NO: 1 - protein, 54 aa, unidentified
TENLKHQPGGGKGSKDNIKHVPGGGSGSLGNIHHKPGGGQGSLDNITHVPGGGN

SEQ ID NO: 2 - DNA, 174 bp, unidentified
  source 1..174: mol_type = other DNA
catatgactgaaaatctgaaacatcaacctggcggcggtaaaggctctaaagataacatcaagcacgttcctggtggcggttctggttccctgggtaacatccatcacaaaccgggtggcggtcaaggtagcctggataatatcactcatgtgccaggtggtggcaatccatgg

SEQ ID NO: 3 - protein, 462 aa, unidentified
KIEEGKLVIWINGDKGYNGLAEVGKKFEKDTGIKVTVEHPDKLEEKFPQVAATGDGPDIIFWAHDRFGGYAQSGLLAEITPDKAFQDKLYPFTWDAVRYNGKLIAYPIAVEALSLIYNKDLLPNPPKTWEEIPALDKELKAKGKSALMFNLQEPYFTWPLIAADGGYAFKYENGKYDIKDVGVDNAGAKAGLTFLVDLIKNKHMNADTDYSIAEAAFNKGETAMTINGPWAWSNIDTSKVNYGVTVLPTFKGQPSKPFVGVLSAGINAASPNKELAKEFLENYLLTDEGLEAVNKDKPLGAVALKSYEEELVKDPRIAATMENAQKGEIMPNIPQMSAFWYAVRTAVINAASGRQTVDEALKDAQTNSSSNNNNNNNNNNLGIEGRISHMTENLKHQPGGGKGSKDNIKHVPGGGSGSLGNIHHKPGGGQGSLDNITHVPGGGNPWAAAISSTDPNSLQVIK

SEQ ID NO: 4 - protein, 444 aa, unidentified
KIEEGKLVIWINGDKGYNGLAEVGKKFEKDTGIKVTVEHPDKLEEKFPQVAATGDGPDIIFWAHDRFGGYAQSGLLAEITPDKAFQDKLYPFTWDAVRYNGKLIAYPIAVEALSLIYNKDLLPNPPKTWEEIPALDKELKAKGKSALMFNLQEPYFTWPLIAADGGYAFKYENGKYDIKDVGVDNAGAKAGLTFLVDLIKNKHMNADTDYSIAEAAFNKGETAMTINGPWAWSNIDTSKVNYGVTVLPTFKGQPSKPFVGVLSAGINAASPNKELAKEFLENYLLTDEGLEAVNKDKPLGAVALKSYEEELVKDPRIAATMENAQKGEIMPNIPQMSAFWYAVRTAVINAASGRQTVDEALKDAQTNSSSGGGGSGGGGSLGIEGRISHMTENLKHQPGGGKGSKDNIKHVPGGGSGSLGNIHHKPGGGQGSLDNITHVPGGGN